European Patent Application EP 4 406 971 A1, published July 31, 2024. Title: ANTI-CD40 ANTIBODY AND USE THEREOF. Applicant: Chia Tai Tianqing Pharmaceutical Group Co., Ltd. The sequence listing filed with the application follows.

SEQUENCE LISTING (82 sequences)

SEQ ID NO: 1 - protein, 10 aa, Mus sp.
GFSLPTSGVH

SEQ ID NO: 2 - protein, 16 aa, Mus sp.
VIWAGGDTNYNSALMS

SEQ ID NO: 3 - protein, 9 aa, synthetic construct
  REGION 1..9: note = HCDR2 of hzA01-1.1, hzA01-1.2, hzA01-2.1, hzA01-2.2 and hzA01-3.1
VIWAGGDTN

SEQ ID NO: 4 - protein, 16 aa, synthetic construct
  REGION 1..16: note = HCDR2 of hzA01-3.3
VIWAGGDTNYNSALKS

SEQ ID NO: 5 - protein, 8 aa, Mus sp.
LGHGHFDV

SEQ ID NO: 6 - protein, 16 aa, Mus sp.
RSSQSLVHSSGNTYLQ

SEQ ID NO: 7 - protein, 7 aa, Mus sp.
KVSNRFS

SEQ ID NO: 8 - protein, 9 aa, Mus sp.
SQTTHVPWT

SEQ ID NO: 9 - protein, 114 aa, Mus sp.
QVQLKESGPGLVAPSQSLSITCTVSGFSLPTSGVHWVRQPPGKGLEWLGVIWAGGDTNYNSALMSRLSISKDNSKSQVFLKMNSLQKDDTAIYYCLGHGHFDVWGAGTTVTVSS

SEQ ID NO: 10 - protein, 114 aa, synthetic construct
  REGION 1..114: note = VH of hzA01-1.1, hzA01-2.1 and hzA01-3.1
QVQLQESGPGLVKPSETLSLTCTVSGFSLPTSGVHWIRQPPGKGLEWIGVIWAGGDTNYNPSLKSRVTISKDNSKNQVFLKLSSVTAADTAVYYCLGHGHFDVWGQGTLVTVSS

SEQ ID NO: 11 - protein, 114 aa, synthetic construct
  REGION 1..114: note = VH of hzA01-1.2 and hzA01-2.2
QVQLVESGGGVVQPGRSLRLSCAASGFSLPTSGVHWVRQAPGKGLEWVAVIWAGGDTNYADSVKGRFTISRDNSKNTVYLQMNSLRAEDTAVYYCLGHGHFDVWGQGTLVTVSS

SEQ ID NO: 12 - protein, 114 aa, synthetic construct
  REGION 1..114: note = VH of hzA01-3.3
QVQLKESGPGLVKPSETLSLTCTVSGFSLPTSGVHWIRQPPGKGLEWIGVIWAGGDTNYNSALKSRVTISKDNSKSQVFLKLSSVTAADTAVYYCLGHGHFDVWGQGTLVTVSS

SEQ ID NO: 13 - protein, 114 aa, synthetic construct
  REGION 1..114: note = VH of hzA01-3.4
QVQLKESGPGLVKPSETLSLTCTVSGFSLPTSGVHWIRQPPGKGLEWIGVIWAGGDTNYNSALMSRVTISKDNSKSQVFLKMSSVTAADTAVYYCLGHGHFDVWGQGTLVTVSS

SEQ ID NO: 14 - protein, 112 aa, Mus sp.
DVVMTQTPLSLPVSLGDQASISCRSSQSLVHSSGNTYLQWYLQKPGQSPGLLIYKVSNRFSGVPDRFSGSGSGTDFTLKISRVEAEDLGVYFCSQTTHVPWTFGGGTKLEIK

SEQ ID NO: 15 - protein, 112 aa, synthetic construct
  REGION 1..112: note = VL of hzA01-1.1 and hzA01-1.2
DIQMTQSPSSLSASVGDRVTITCRSSQSLVHSSGNTYLQWYQQKPGKAPGLLIYKVSNRFSGVPSRFSGSGSGTDFTLTISSLQPEDFATYYCSQTTHVPWTFGQGTKVEIK

SEQ ID NO: 16 - protein, 112 aa, synthetic construct
  REGION 1..112: note = VL of hzA01-2.1 and hzA01-2.2
EIVLTQSPGTLSLSPGERATLSCRSSQSLVHSSGNTYLQWYQQKPGQAPRLLIYKVSNRFSGIPDRFSGSGSGTDFTLTISRLEPEDFAVYYCSQTTHVPWTFGQGTKVEIK

SEQ ID NO: 17 - protein, 112 aa, synthetic construct
  REGION 1..112: note = VL of hzA01-3.1, hzA01-3.3 and hzA01-3.4
DVVMTQSPLSLPVTLGQPASISCRSSQSLVHSSGNTYLQWYLQRPGQSPGLLIYKVSNRFSGVPDRFSGSGSGTDFTLKISRVEAEDVGVYYCSQTTHVPWTFGQGTKLEIK

SEQ ID NO: 18 - protein, 10 aa, Mus sp.
GFSLTSSGVH

SEQ ID NO: 19 - protein, 16 aa, Mus sp.
VIWAGGDTSYNSALMS

SEQ ID NO: 20 - protein, 8 aa, Mus sp.
LGHGHLDV

SEQ ID NO: 21 - protein, 20 aa, Mus sp.
RSSQSLVHSSGNTYLHWYLQ

SEQ ID NO: 22 - protein, 114 aa, Mus sp.
QVQLKESGPGLVAPSQSLSITCTVSGFSLTSSGVHWVRQPPGKGLEWLGVIWAGGDTSYNSALMSRLSISKDNSKSQVFLKMNSLQTDDTAMYYCLGHGHLDVWGAGTTVTVSS

SEQ ID NO: 23 - protein, 112 aa, Mus sp.
DVVMTQTPLSLPVSLGDQASISCRSSQSLVHSSGNTYLHWYLQKPGQSPGLLIYKVSNRFSGVPDRFSGSGSGTDFTLKISRVEAEDLGVYFCSQTTHVPWTFGGGTKLEIK

SEQ ID NO: 24 - protein, 11 aa, Mus sp.
GYSITSDYSWH

SEQ ID NO: 25 - protein, 16 aa, Mus sp.
YIYSSGHTYYNPSLKS

SEQ ID NO: 26 - protein, 10 aa, Mus sp.
YYYGRSYFDN

SEQ ID NO: 27 - protein, 10 aa, Mus sp.
SASSSVNYMH

SEQ ID NO: 28 - protein, 7 aa, Mus sp.
DTSKLAS

SEQ ID NO: 29 - protein, 9 aa, Mus sp.
QQWSSNPLT

SEQ ID NO: 30 - protein, 119 aa, Mus sp.
DVQLQESGPDRVKPSQSLSLTCTVTGYSITSDYSWHWIRQFPGNKLEWMGYIYSSGHTYYNPSLKSRISFTRDTSKNQFFLQLNSVTTEDTATYYCAIYYYGRSYFDNWGRGTTLTVSS

SEQ ID NO: 31 - protein, 106 aa, Mus sp.
QIVLTQSPAIMSASPGEKVTLTCSASSSVNYMHWYQQKSGTSPKRWIYDTSKLASGVPARFSGSGSGTSYSLTISSMEAEDAATYYCQQWSSNPLTFGAGTKLELK

SEQ ID NO: 32 - protein, 10 aa, Mus sp.
GYTFTNYGMN

SEQ ID NO: 33 - protein, 17 aa, Mus sp.
WINPYTGEPTYADDFKG

SEQ ID NO: 34 - protein, 6 aa, Mus sp.
KPPFDY

SEQ ID NO: 35 - protein, 16 aa, Mus sp.
RSSKSLLHSNGNTYLY

SEQ ID NO: 36 - protein, 7 aa, Mus sp.
RVSNLAS

SEQ ID NO: 37 - protein, 9 aa, Mus sp.
MQHVEYPFT

SEQ ID NO: 38 - protein, 115 aa, Mus sp.
QIQLVQSGPELKKPGETVKISCKASGYTFTNYGMNWVKQAPGKGLKWMGWINPYTGEPTYADDFKGRFAFSVETSASTAYLQINNLKNEDTATYFCARKPPFDYWGQGTTLTVSS

SEQ ID NO: 39 - protein, 112 aa, Mus sp.
DIVMTQAAPSVPVTPGESVSISCRSSKSLLHSNGNTYLYWFLQRPGQSPQILIYRVSNLASGVPDRFSGSGSGTAFTLRISRVEAEDVGVYYCMQHVEYPFTFGSGTKLEIK

SEQ ID NO: 40 - protein, 10 aa, Mus sp.
GYTFTSYVMY

SEQ ID NO: 41 - protein, 17 aa, Mus sp.
YVNPYNDGTNYNEKFKG

SEQ ID NO: 42 - protein, 5 aa, Mus sp.
GAMDY

SEQ ID NO: 43 - protein, 16 aa, Mus sp.
RSSKSLLHSQGNTYLY

SEQ ID NO: 44 - protein, 114 aa, Mus sp.
EVQLQQSGPELVKPGASVKMSCKASGYTFTSYVMYWVKQKPGQGLEWIGYVNPYNDGTNYNEKFKGKATLTSDKSSSTAYMELSSLTSEDSAVYYCARGAMDYWGQGTSVTVSS

SEQ ID NO: 45 - protein, 112 aa, Mus sp.
DIVMTQAAPSVPVTPGESVSISCRSSKSLLHSQGNTYLYWFLQRPGQSPQILIYRVSNLASGVPDRFSGSGSGTAFTLRISRVEAEDVGVYYCMQHVEYPFTFGSGTKLEIK

SEQ ID NO: 46 - protein, 10 aa, Mus sp.
GFTFSDFYME

SEQ ID NO: 47 - protein, 19 aa, Mus sp.
ASRDKANDYTTEYSPSVQG

SEQ ID NO: 48 - protein, 10 aa, Mus sp.
DVGRSYALDY

SEQ ID NO: 49 - protein, 10 aa, Mus sp.
SASSSVTYMH

SEQ ID NO: 50 - protein, 7 aa, Mus sp.
VTSKLAS

SEQ ID NO: 51 - protein, 9 aa, Mus sp.
QQWSRKPPT

SEQ ID NO: 52 - protein, 121 aa, Mus sp.
EVKLVESGGGLVQPGGSLRLSCATSGFTFSDFYMEWVRQPPGKRLEWIAASRDKANDYTTEYSPSVQGRFIVSRDSSQSILYLQMNALRTEDTAIYYCARDVGRSYALDYWGQGTSVTVSS

SEQ ID NO: 53 - protein, 106 aa, Mus sp.
QVVLTQSPAIMSASPGEKVTMTCSASSSVTYMHWYQQKSGTSPKRWIYVTSKLASGVPTRFSGSGSGTSYSLTISSMEAEDAATYYCQQWSRKPPTFGAGTKLELK

SEQ ID NO: 54 - protein, 327 aa, synthetic construct
  REGION 1..327: note = Heavy chain constant region of chimeric and humanized antibodies
ASTKGPSVFPLAPCSRSTSESTAALGCLVKDYFPEPVTVSWNSGALTSGVHTFPAVLQSSGLYSLSSVVTVPSSSLGTKTYTCNVDHKPSNTKVDKRVESKYGPPCPPCPAPEFEGGPSVFLFPPKPKDTLMISRTPEVTCVVVDVSQEDPEVQFNWYVDGVEVHNAKTKPREEQFNSTYRVVSVLTVLHQDWLNGKEYKCKVSNKGLPSSIEKTISKAKGQPREPQVYTLPPSQEEMTKNQVSLTCLVKGFYPSDIAVEWESNGQPENNYKTTPPVLDSDGSFFLYSRLTVDKSRWQEGNVFSCSVMHEALHNHYTQKSLSLSLGK

SEQ ID NO: 55 - protein, 327 aa, Homo sapiens
ASTKGPSVFPLAPCSRSTSESTAALGCLVKDYFPEPVTVSWNSGALTSGVHTFPAVLQSSGLYSLSSVVTVPSSSLGTKTYTCNVDHKPSNTKVDKRVESKYGPPCPSCPAPEFLGGPSVFLFPPKPKDTLMISRTPEVTCVVVDVSQEDPEVQFNWYVDGVEVHNAKTKPREEQFNSTYRVVSVLTVLHQDWLNGKEYKCKVSNKGLPSSIEKTISKAKGQPREPQVYTLPPSQEEMTKNQVSLTCLVKGFYPSDIAVEWESNGQPENNYKTTPPVLDSDGSFFLYSRLTVDKSRWQEGNVFSCSVMHEALHNHYTQKSLSLSLGK

SEQ ID NO: 56 - protein, 327 aa, synthetic construct
  REGION 1..327: note = IgG4 heavy chain constant region with 1 amino acid mutation (S228P)
ASTKGPSVFPLAPCSRSTSESTAALGCLVKDYFPEPVTVSWNSGALTSGVHTFPAVLQSSGLYSLSSVVTVPSSSLGTKTYTCNVDHKPSNTKVDKRVESKYGPPCPPCPAPEFLGGPSVFLFPPKPKDTLMISRTPEVTCVVVDVSQEDPEVQFNWYVDGVEVHNAKTKPREEQFNSTYRVVSVLTVLHQDWLNGKEYKCKVSNKGLPSSIEKTISKAKGQPREPQVYTLPPSQEEMTKNQVSLTCLVKGFYPSDIAVEWESNGQPENNYKTTPPVLDSDGSFFLYSRLTVDKSRWQEGNVFSCSVMHEALHNHYTQKSLSLSLGK

SEQ ID NO: 57 - protein, 107 aa, Homo sapiens [sequence omitted]

SEQ ID NO: 58 - protein, 450 aa, synthetic construct
  REGION 1..450: note = Heavy chain of Iscalimab(CFZ533)
QVQLVESGGGVVQPGRSLRLSCAASGFTFSSYGMHWVRQAPGKGLEWVAVISYEESNRYHADSVKGRFTISRDNSKITLYLQMNSLRTEDTAVYYCARDGGIAAPGPDYWGQGTLVTVSSASTKGPSVFPLAPSSKSTSGGTAALGCLVKDYFPEPVTVSWNSGALTSGVHTFPAVLQSSGLYSLSSVVTVPSSSLGTQTYICNVNHKPSNTKVDKRVEPKSCDKTHTCPPCPAPELLGGPSVFLFPPKPKDTLMISRTPEVTCVVVDVSHEDPEVKFNWYVDGVEVHNAKTKPREEQYASTYRVVSVLTVLHQDWLNGKEYKCKVSNKALPAPIEKTISKAKGQPREPQVYTLPPSREEMTKNQVSLTCLVKGFYPSDIAVEWESNGQPENNYKTTPPVLDSDGSFFLYSKLTVDKSRWQQGNVFSCSVMHEALHNHYTQKSLSLSPGK

SEQ ID NO: 59 - protein, 219 aa, synthetic construct
  REGION 1..219: note = Light chain of Iscalimab(CFZ533)
DIVMTQSPLSLTVTPGEPASISCRSSQSLLYSNGYNYLDWYLQKPGQSPQVLISLGSNRASGVPDRFSGSGSGTDFTLKISRVEAEDVGVYYCMQARQTPFTFGPGTKVDIRRTVAAPSVFIFPPSDEQLKSGTASVVCLLNNFYPREAKVQWKVDNALQSGNSQESVTEQDSKDSTYSLSSTLTLSKADYEKHKVYACEVTHQGLSSPVTKSFNRGEC

SEQ ID NO: 60 - protein, 452 aa, synthetic construct
  REGION 1..452: note = Heavy chain of CP-870893
QVQLVQSGAEVKKPGASVKVSCKASGYTFTGYYMHWVRQAPGQGLEWMGWINPDSGGTNYAQKFQGRVTMTRDTSISTAYMELNRLRSDDTAVYYCARDQPLGYCTNGVCSYFDYWGQGTLVTVSSASTKGPSVFPLAPCSRSTSESTAALGCLVKDYFPEPVTVSWNSGALTSGVHTFPAVLQSSGLYSLSSVVTVPSSNFGTQTYTCNVDHKPSNTKVDKTVERKCCVECPPCPAPPVAGPSVFLFPPKPKDTLMISRTPEVTCVVVDVSHEDPEVQFNWYVDGVEVHNAKTKPREEQFNSTFRVVSVLTVVHQDWLNGKEYKCKVSNKGLPAPIEKTISKTKGQPREPQVYTLPPSREEMTKNQVSLTCLVKGFYPSDIAVEWESNGQPENNYKTTPPMLDSDGSFFLYSKLTVDKSRWQQGNVFSCSVMHEALHNHYTQKSLSLSPGK

SEQ ID NO: 61 - protein, 214 aa, synthetic construct
  REGION 1..214: note = Light chain of CP-870893
DIQMTQSPSSVSASVGDRVTITCRASQGIYSWLAWYQQKPGKAPNLLIYTASTLQSGVPSRFSGSGSGTDFTLTISSLQPEDFATYYCQQANIFPLTFGGGTKVEIKRTVAAPSVFIFPPSDEQLKSGTASVVCLLNNFYPREAKVQWKVDNALQSGNSQESVTEQDSKDSTYSLSSTLTLSKADYEKHKVYACEVTHQGLSSPVTKSFNRGEC

SEQ ID NO: 62 - protein, 277 aa, Homo sapiens
MVRLPLQCVLWGCLLTAVHPEPPTACREKQYLINSQCCSLCQPGQKLVSDCTEFTETECLPCGESEFLDTWNRETHCHQHKYCDPNLGLRVQQKGTSETDTICTCEEGWHCTSEACESCVLHRSCSPGFGVKQIATGVSDTICEPCPVGFFSNVSSAFEKCHPWTSCETKDLVVQQAGTNKTDVVCGPQDRLRALVVIPIIFGILFAILLVLVFIKKVAKKPTNKAPHPKQEPQEINFPDDLPGSNTAAPVQETLHGCQPVTQEDGKESRISVQERQ

SEQ ID NO: 63 - protein, 278 aa, Macaca fascicularis
MVRLPLQCVLWGCLLTAVYPEPPTACREKQYLINSQCCSLCQPGQKLVSDCTEFTETECLPCGESEFLDTWNRETRCHQHKYCDPNLGLRVQQKGTSETDTICTCEEGLHCTSESCESCVPHRSCLPGFGVKQIATGVSDTICEPCPVGFFSNVSSAFEKCRPWTSCETKDLVVQQAGTNKTDVVCGPQDRQRALVVIPICLGILFVILLLVLVFIKKVAKKPNDKVPHPKQEPQEINFPDDLPGSNPAAPVQETLHGCQPVTQEDGKESRISVQERQ

SEQ ID NO: 64 - protein, 426 aa, synthetic construct
  REGION 1..426: note = human CD40-mFc (hCD40-mFc)
MVRLPLQCVLWGCLLTAVHPEPPTACREKQYLINSQCCSLCQPGQKLVSDCTEFTETECLPCGESEFLDTWNRETHCHQHKYCDPNLGLRVQQKGTSETDTICTCEEGWHCTSEACESCVLHRSCSPGFGVKQIATGVSDTICEPCPVGFFSNVSSAFEKCHPWTSCETKDLVVQQAGTNKTDVVCGPQDRLREPRGPTIKPCPPCKCPAPNLLGGPSVFIFPPKIKDVLMISLSPIVTCVVVDVSEDDPDVQISWFVNNVEVHTAQTQTHREDYNSTLRVVSALPIQHQDWMSGKEFKCKVNNKDLPAPIERTISKPKGSVRAPQVYVLPPPEEEMTKKQVTLTCMVTDFMPEDIYVEWTNNGKTELNYKNTEPVLDSDGSYFMYSKLRVEKKNWVERNSYSCSVVHEGLHNHHTTKSFSRTPGK

SEQ ID NO: 65 - protein, 426 aa, synthetic construct
  REGION 1..426: note = Cynomolgus monkey CD40-mFc (cynoCD40-mFc)
MVRLPLQCVLWGCLLTAVYPEPPTACREKQYLINSQCCSLCQPGQKLVSDCTEFTETECLPCGESEFLDTWNRETRCHQHKYCDPNLGLRVQQKGTSETDTICTCEEGLHCTSESCESCVPHRSCLPGFGVKQIATGVSDTICEPCPVGFFSNVSSAFEKCRPWTSCETKDLVVQQAGTNKTDVVCGPQDRQREPRGPTIKPCPPCKCPAPNLLGGPSVFIFPPKIKDVLMISLSPIVTCVVVDVSEDDPDVQISWFVNNVEVHTAQTQTHREDYNSTLRVVSALPIQHQDWMSGKEFKCKVNNKDLPAPIERTISKPKGSVRAPQVYVLPPPEEEMTKKQVTLTCMVTDFMPEDIYVEWTNNGKTELNYKNTEPVLDSDGSYFMYSKLRVEKKNWVERNSYSCSVVHEGLHNHHTTKSFSRTPGK

SEQ ID NO: 66 - protein, 261 aa, Homo sapiens
MIETYNQTSPRSAATGLPISMKIFMYLLTVFLITQMIGSALFAVYLHRRLDKIEDERNLHEDFVFMKTIQRCNTGERSLSLLNCEEIKSQFEGFVKDIMLNKEETKKENSFEMQKGDQNPQIAAHVISEASSKTTSVLQWAEKGYYTMSNNLVTLENGKQLTVKRQGLYYIYAQVTFCSNREASSQAPFIASLCLKSPGRFERILLRAANTHSSAKPCGQQSIHLGGVFELQPGASVFVNVTDPSQVSHGTGFTSFGLLKL

SEQ ID NO: 67 - protein, 261 aa, Macaca fascicularis
MIETYNQPSPRSAATGLPVRMKIFMYLLTIFLITQMIGSALFAVYLHRRLDKIEDERNLHEDFVFMKTIQRCNTGEKSLSLLNCEEIKSQFEGFVKDIMLNKEEKKKENSFEMQKGDQNPQIAAHVISEASSKTTSVLQWAEKGYYTMSNNLVTLENGKQLTVKRQGLYYIYAQVTFCSNREASSQAPFIASLCLKSPGRFERILLRAANTHSSAKPCGQQSIHLGGVFELQPGASVFVNVTDPSQVSHGTGFTSFGLLKL

SEQ ID NO: 68 - DNA, 342 bp, synthetic construct
  gene 1..342: note = VH of mouse and chimeric A01
  source 1..342: mol_type = other DNA
caagttcagttgaaagaatccgggcctggtctcgttgctccttcccagagtctctccataacctgcacagtgagcggcttttctttgcccaccagtggagtgcactgggtgcgacagccacctggaaaaggtcttgagtggttgggtgtgatctgggcaggtggggacaccaattataactccgccctgatgagccgcctctccatctccaaggataattctaagtctcaggtgttcctgaaaatgaactcccttcagaaggacgataccgccatctactattgcctgggacacgggcattttgacgtgtggggtgctgggacaaccgtgaccgtgagctct

SEQ ID NO: 69 - DNA, 342 bp, synthetic construct
  gene 1..342: note = VH of hzA01-1.1, hzA01-2.1 and hzA01-3.1
  source 1..342: mol_type = other DNA
caagtgcaactgcaggaatctggcccaggccttgttaaaccatctgaaaccctgagcttgacttgcactgtgagtggcttcagcttgccaacttccggtgtgcactggattagacagcccccaggcaaagggctggaatggatcggcgtgatttgggccggcggagacaccaattacaacccaagcctgaagagtcgggtgaccatctccaaggataattccaagaaccaagtgtttctcaaactgtcctctgtgacggctgctgataccgctgtctactactgtctcggccacgggcatttcgacgtttgggggcagggtacattggtgaccgtaagcagc

SEQ ID NO: 70 - DNA, 342 bp, synthetic construct
  gene 1..342: note = VH of hzA01-1.2 and hzA01-2.2
  source 1..342: mol_type = other DNA
caagttcagctcgtagaatctggtggtggagtggttcaaccaggcaggagcttgaggctgtcatgtgccgcatctgggttctcactccccacctctggcgtgcactgggttagacaggctccaggaaaggggctggaatgggtcgctgtgatttgggcaggaggagacactaactatgccgactctgttaagggacggtttacaatcagcagagataactcaaaaaacaccgtgtacttgcagatgaattcactgagggctgaagacacagcggtgtattactgcctcggtcacggccacttcgatgtctggggccagggtacacttgtgactgtcagcagc

SEQ ID NO: 71 - DNA, 342 bp, synthetic construct
  gene 1..342: note = VH of hzA01-3.3
  source 1..342: mol_type = other DNA
caggtgcagctcaaagaaagtgggcctgggttggtcaaaccttctgagaccctgagtctgacctgcaccgtatcagggtttagcttgccaactagcggcgtacattggatcaggcagccaccaggcaagggactcgaatggatcggcgtgatttgggccgggggcgataccaattacaattcagctctcaagtcccgcgtcaccatctcaaaagacaacagtaaaagccaggtcttcctgaagctgtccagtgtgacagctgctgacaccgccgtgtactattgtctggggcacggacatttcgacgtgtggggccaaggcaccctggtgacagtgagcagc

SEQ ID NO: 72 - DNA, 342 bp, synthetic construct
  gene 1..342: note = VH of hzA01-3.4
  source 1..342: mol_type = other DNA
caggtgcagttgaaagaatctggacccgggcttgtcaagccatcagaaactctgagtcttacctgcaccgtttcagggttttccctcccaacatccggcgttcactggattcggcagcctcctgggaagggactggaatggattggcgtcatttgggcaggaggagatacaaattataactcagccctgatgtcccgggtgaccatctcaaaggataactccaaatcccaggtttttctgaagatgtccagcgtaaccgccgcagatacagccgtctactattgcctgggtcatggacatttcgatgtgtggggccagggaaccctcgtcactgtctccagt

SEQ ID NO: 73 - DNA, 336 bp, synthetic construct
  gene 1..336: note = VL of mouse and chimeric A01
  source 1..336: mol_type = other DNA
gatgttgtgatgacacagacacctctgtccttgccagtcagcttgggagatcaggcttcaatcagctgcaggtcctctcagagtctcgtacattcatcaggaaacacctacctccagtggtacttgcagaagccaggccaatctcctggactgctgatctacaaggtctccaataggttttctggagtgcccgataggttcagcggcagcggtagcggcacagactttactctgaaaatttcacgagtggaagcagaagatttgggggtctatttttgctcccagacaactcacgtgccatggacctttggcggagggactaaactggagatcaag

SEQ ID NO: 74 - DNA, 336 bp, synthetic construct
  gene 1..336: note = VL of hzA01-1.1 and hzA01-1.2
  source 1..336: mol_type = other DNA
gatatccagatgacccaatcaccctctagcctcagtgcaagtgtgggagatagggtaactatcacctgcagaagtagtcaatcactggtgcacagttccggaaacacctacctgcagtggtaccagcagaagcctgggaaggcaccaggcctgctgatatacaaagttagtaacaggttttccggggtgccaagccgatttagcggatctggctccgggacagacttcaccctgaccatcagctccctgcagccagaagactttgccacctattattgcagccagactacacacgtaccttggacctttggacagggtacaaaagtggagataaag

SEQ ID NO: 75 - DNA, 336 bp, synthetic construct
  gene 1..336: note = VL of hzA01-2.1 and hzA01-2.2
  source 1..336: mol_type = other DNA
gagattgtccttactcagtctcctggcactctgagcttgtcacctggagagcgagctactttgagctgccggtcatcacagtcattggtccacagctcaggcaacacatacctccagtggtaccaacagaagccaggacaggctccacgcctcctgatctacaaggtcagcaatcggtttagcggaatcccagaccgcttttcaggcagcggtagcggcacagattttactttgactatctctagactggagcccgaggattttgccgtgtactattgcagccagacaactcatgtgccttggactttcggccagggaacaaaggtggagatcaaa

SEQ ID NO: 76 - DNA, 336 bp, synthetic construct
  gene 1..336: note = VL of hzA01-3.1, hzA01-3.3 and hzA01-3.4
  source 1..336: mol_type = other DNA
gatgttgtaatgactcagagtccactgtctcttccagtcaccctggggcagcctgcatctatttcctgccggagctcacaaagcctggtgcactccagtggaaatacctacctgcagtggtatttgcaaaggcccggacagtctccaggtctgttgatatataaggtatccaataggttcagtggggtgccagaccgattttctggatcaggttcaggcaccgattttaccctcaagatctcaagagtggaagccgaagacgtgggcgtctactactgcagccagactacccacgtgccttggacctttggacaggggaccaaactggagattaaa

SEQ ID NO: 77 - DNA, 981 bp, synthetic construct
  source 1..981: mol_type = other DNA
  gene 1..981: note = Heavy chain constant region of chimeric and humanized antibodies
gcttcaacaaaaggaccctctgtttttcctctcgcaccctgttcccgcagcacaagcgagtctactgccgcactcggctgtctggttaaagactattttcctgagcccgtgaccgtgagttggaacagcggtgccctgacctcaggagtgcatacctttccggcagtgttgcagtcatcaggtctgtatagcctgagcagtgttgtgacagtgccctcaagtagcttgggcacaaagacatatacttgtaacgtcgatcataagccttccaacacaaaggtggacaagagggtggagtccaagtacggaccaccttgccctccatgtcctgcaccagagttcgaaggcggcccttctgtcttcttgtttcccccaaagccgaaggataccttgatgatctctagaacgccagaagtgacatgcgtagtggttgacgtaagccaggaagacccagaagtgcagtttaattggtatgtggacggggttgaggttcataacgcgaagactaagcctcgagaagaacaattcaattccacttatagagtggtgtccgtgcttaccgtgctgcatcaagattggttgaatgggaaagagtacaagtgtaaggtgtccaataaaggcctcccatcttcaattgaaaagacaatttccaaagccaagggacaaccccgagagccacaggtctacaccctgcctccttcccaggaagagatgaccaagaatcaggtttcattgacatgcctggtcaaaggcttctaccccagcgacatcgctgttgagtgggagtcaaatggtcaaccagaaaacaactataaaaccacccctcccgtgctggattcagacggttctttttttctgtattccagactcacagtcgacaagagcagatggcaggaagggaacgtcttttcctgttcagtgatgcacgaggctctgcataatcactacacccaaaagtccttgtctctgagtttgggcaaa

SEQ ID NO: 78 - DNA, 321 bp, synthetic construct
  source 1..321: mol_type = other DNA
  gene 1..321: note = Light chain constant region of chimeric and humanized antibodies
cgcacagtggctgctccctcagtatttatctttcctccaagcgacgagcaactgaagtctgggacggcttccgtggtgtgtctgctgaataatttttatcctagagaagctaaggtccagtggaaagtagacaatgccttgcagagtggaaacagccaggagtccgtgacggaacaggactccaaagattccacttactccttgtcctcaacccttactttgagcaaagccgattatgaaaagcataaggtctacgcctgcgaggtgacccaccaggggttgagttcacctgtcaccaaaagcttcaaccgaggggaatgt

SEQ ID NO: 79 - protein, 5 aa, Mus sp.
TSGVH

SEQ ID NO: 80 - protein, 16 aa, synthetic construct
  REGION 1..16: note = HCDR2 of hzA01-1.1, hzA01-2.1 and hzA01-3.1 (Kabat numbering)
VIWAGGDTNYNPSLKS

SEQ ID NO: 81 - protein, 16 aa, synthetic construct
  REGION 1..16: note = HCDR2 of hzA01-1.2 and hzA01-2.2 (Kabat numbering)
VIWAGGDTNYADSVKG

SEQ ID NO: 82 - protein, 6 aa, Mus sp.
HGHFDV